European Patent Specification EP 3 842 041 B1, published May 21, 2025. Title: Composition for Treating and Preventing Gingivoperiodontitis or Periimplantitis and Proxabrush Coated with the Composition. Applicant: Nano Intelligent Biomedical Engineering Corporation. co. Ltd. The sequence listing filed with the application follows.

SEQUENCE LISTING (4 sequences)

SEQ ID NO: 1 - protein, 15 aa, Artificial Sequence
  Antimicrobial Peptide
GKCSTRGRKCCRRKK

SEQ ID NO: 2 - protein, 15 aa, Artificial Sequence
  Antimicrobial Peptide
GKSSTRGRKSCRRKK

SEQ ID NO: 3 - protein, 15 aa, Artificial Sequence
  Antimicrobial Peptide
GKCSTRGRKSSRRKK

SEQ ID NO: 4 - protein, 15 aa, Artificial Sequence
  Antimicrobial Peptide
GKSSTRGRKCSRRKK